European Patent Specification EP 3 872 067 B1, published June 18, 2025. Title: PROLINE-LOCKED STAPLED PEPTIDES AND USES THEREOF. Applicant: PRESIDENT AND FELLOWS OF HARVARD COLLEGE. The sequence listing filed with the application follows.

SEQUENCE LISTING (38 sequences)

SEQ ID NO: 1 - protein, 14 aa, Artificial Sequence
  Synthetic polypeptide
PAALKRARNTEAAW

SEQ ID NO: 2 - protein, 14 aa, Artificial Sequence
  Synthetic polypeptide
  misc_feature (1)..(1): Xaa is a modified Pro
  misc_feature (4)..(4): Xaa is a modified Ser
XAAXKRARNTEAAW

SEQ ID NO: 3 - protein, 26 aa, Artificial Sequence
  Synthetic polypeptide
MKDPAALKRARNTEAARRSRARKLQR

SEQ ID NO: 4 - protein, 32 aa, Artificial Sequence
  Synthetic polypeptide
MKQLEDKVEELLSKNYHLENEVARLKKLVGER

SEQ ID NO: 5 - protein, 14 aa, Artificial Sequence
  Synthetic polypeptide
  misc_feature (1)..(1): Xaa is a modified Pro
XAALKRARNTEAAW

SEQ ID NO: 6 - protein, 14 aa, Artificial Sequence
  Synthetic polypeptide
  misc_feature (1)..(1): Xaa is a modified Pro
XAALKRARNTEAAW

SEQ ID NO: 7 - protein, 14 aa, Artificial Sequence
  Synthetic polypeptide
  misc_feature (1)..(1): Xaa is a modified Pro
  misc_feature (4)..(4): Xaa is a modified Arg
XAAXKRARNTEAAW

SEQ ID NO: 8 - protein, 14 aa, Artificial Sequence
  Synthetic polypeptide
  misc_feature (1)..(1): Xaa is a modified Pro
  misc_feature (4)..(4): Xaa is a modified Ser
XAAXKRARNTEAAW

SEQ ID NO: 9 - protein, 14 aa, Artificial Sequence
  Synthetic polypeptide
  misc_feature (1)..(1): Xaa is a modified Pro
  misc_feature (4)..(4): Xaa is a modified Arg
XAAXKRARNTEAAW

SEQ ID NO: 10 - protein, 14 aa, Artificial Sequence
  Synthetic polypeptide
  misc_feature (1)..(1): Xaa is a modified Pro
XAALKRARNTEAAW

SEQ ID NO: 11 - protein, 14 aa, Artificial Sequence
  Synthetic polypeptide
  misc_feature (1)..(1): Xaa is a modified Pro
  misc_feature (4)..(4): Xaa is a modified Ser
XAAXKRARNTEAAW

SEQ ID NO: 12 - protein, 14 aa, Artificial Sequence
  Synthetic polypeptide
  misc_feature (1)..(1): Xaa is a modified Pro
  misc_feature (4)..(4): Xaa is a modified Arg
XAAXKRARNTEAAW

SEQ ID NO: 13 - protein, 14 aa, Artificial Sequence
  Synthetic polypeptide
  misc_feature (1)..(1): Xaa is a modified Pro
  misc_feature (4)..(4): Xaa is a modified Ser
XAAXKRARNTEAAW

SEQ ID NO: 14 - protein, 14 aa, Artificial Sequence
  Synthetic polypeptide
  misc_feature (1)..(1): Xaa is a modified Arg
  misc_feature (4)..(4): Xaa is a modified Ser
XAAXKRARNTEAAW

SEQ ID NO: 15 - protein, 8 aa, Artificial Sequence
  Synthetic polypeptide
PAAAAAAW

SEQ ID NO: 16 - protein, 8 aa, Artificial Sequence
  Synthetic polypeptide
  misc_feature (1)..(1): Xaa is a modified Pro
XAAAAAAW

SEQ ID NO: 17 - protein, 8 aa, Artificial Sequence
  Synthetic polypeptide
  misc_feature (1)..(1): Xaa is a modified Pro
  misc_feature (4)..(4): Xaa is a modified Ser
XAAXAAAW

SEQ ID NO: 18 - protein, 8 aa, Artificial Sequence
  Synthetic polypeptide
  misc_feature (1)..(1): Xaa is a modified Pro
  misc_feature (4)..(4): Xaa is a modified Ser
XAAXAAAW

SEQ ID NO: 19 - protein, 14 aa, Artificial Sequence
  Synthetic polypeptide
  misc_feature (1)..(1): Xaa is a modified Pro
  misc_feature (4)..(4): Xaa is a modified Ser
XAAXKRARNTEAAW

SEQ ID NO: 20 - protein, 14 aa, Artificial Sequence
  Synthetic polypeptide
  misc_feature (1)..(1): Xaa is a modified Pro
  misc_feature (4)..(4): Xaa is a modified Ser
XAAXKRARNTEAAW

SEQ ID NO: 21 - protein, 14 aa, Artificial Sequence
  Synthetic polypeptide
  misc_feature (1)..(1): Xaa is a modified Arg
  misc_feature (4)..(4): Xaa is a modified Ser
XAAXKRARNTEAAW

SEQ ID NO: 22 - protein, 24 aa, Artificial Sequence
  Synthetic polypeptide
PAALKRARNTEAARRSRARKLQRW

SEQ ID NO: 23 - protein, 24 aa, Artificial Sequence
  Synthetic polypeptide
  misc_feature (1)..(1): Xaa is a modified Pro
  misc_feature (4)..(4): Xaa is a modified Ser
XAAXKRARNTEAARRSRARKLQRW

SEQ ID NO: 24 - protein, 5 aa, Artificial Sequence
  Synthetic polypeptide
PAALW

SEQ ID NO: 25 - protein, 5 aa, Artificial Sequence
  Synthetic polypeptide
  misc_feature (1)..(1): Xaa is a modified Pro
  misc_feature (4)..(4): Xaa is a modified Ser
XAAXW

SEQ ID NO: 26 - protein, 14 aa, Artificial Sequence
  Synthetic polypeptide
  misc_feature (1)..(1): Xaa is a modified Ser
  misc_feature (5)..(5): Xaa is a modified Ser
XAALXRARNTEAAW

SEQ ID NO: 27 - protein, 6 aa, Artificial Sequence
  Synthetic polypeptide
NTEAAW

SEQ ID NO: 28 - protein, 6 aa, Artificial Sequence
  Synthetic polypeptide
  misc_feature (1)..(1): Xaa is a modified Pro
  misc_feature (4)..(4): Xaa is a modified Ser
XAAXKR

SEQ ID NO: 29 - protein, 14 aa, Artificial Sequence
  Synthetic polypeptide
  misc_feature (1)..(1): Xaa is a modified Pro
  misc_feature (7)..(7): Xaa is a modified Ser
XAALKRXRNTEAAW

SEQ ID NO: 30 - protein, 14 aa, Artificial Sequence
  Synthetic polypeptide
  misc_feature (1)..(1): Xaa is a modified Pro
  misc_feature (7)..(7): Xaa is a modified Arg
XAALKRXRNTEAAW

SEQ ID NO: 31 - protein, 14 aa, Artificial Sequence
  Synthetic polypeptide
  misc_feature (1)..(1): Xaa is a modified Pro
  misc_feature (8)..(8): Xaa is a modified Ser
XAALKRAXNTEAAW

SEQ ID NO: 32 - protein, 14 aa, Artificial Sequence
  Synthetic polypeptide
  misc_feature (1)..(1): Xaa is a modified Pro
  misc_feature (8)..(8): Xaa is a modified Arg
XAALKRAXNTEAAW

SEQ ID NO: 33 - protein, 14 aa, Artificial Sequence
  Synthetic polypeptide
  misc_feature (1)..(1): Xaa is a modified Arg
  misc_feature (8)..(8): Xaa is a modified Ser
XAALKRAXNTEAAW

SEQ ID NO: 34 - protein, 14 aa, Artificial Sequence
  Synthetic polypeptide
  misc_feature (1)..(1): Xaa is a modified Pro
  misc_feature (8)..(8): Xaa is a modified Ser
XAALKRAXNTEAAW

SEQ ID NO: 35 - protein, 14 aa, Artificial Sequence
  Synthetic polypeptide
  misc_feature (1)..(1): Xaa is a modified Pro
  misc_feature (4)..(4): Xaa is synthetic amino acid
  misc_feature (7)..(7): Xaa is a modified Ser
XAAXKRXRNTEAAW

SEQ ID NO: 36 - protein, 14 aa, Artificial Sequence
  Synthetic polypeptide
  misc_feature (1)..(1): Xaa is a modified Pro
  misc_feature (4)..(4): Xaa is synthetic amino acid
  misc_feature (8)..(8): Xaa is a modified Arg
XAAXKRAXNTEAAW

SEQ ID NO: 37 - protein, 14 aa, Artificial Sequence
  Synthetic polypeptide
  misc_feature (1)..(1): Xaa is a modified Pro
  misc_feature (4)..(4): Xaa is synthetic amino acid
  misc_feature (11)..(11): Xaa is a modified Ser
XAAXKRARNTXAAW

SEQ ID NO: 38 - protein, 14 aa, Artificial Sequence
  Synthetic polypeptide
  misc_feature (1)..(1): Xaa is a modified Pro
  misc_feature (4)..(4): Xaa is a modified Ser
  misc_feature (12)..(12): Xaa is a modified Arg
XAAXKRARNTEXAW